European Patent Specification EP 3 589 735 B1, published July 10, 2024. Title: CONJUGATES COMPRISING OCULAR ANGIOGENESSIS GROWTH FACTOR APTAMERS AND USES THEREOF IN THE DETECTION AND TREATMENT OF OPHTHALMOLOGICAL ANGIOGENESIS INDICATIONS. Applicant: Yissum Research Development Company of the Hebrew University of Jerusalem Ltd. The sequence listing filed with the application follows.

SEQUENCE LISTING (4 sequences)

SEQ ID NO: 1 - DNA, 12 bp, Artificial Sequence
  single-stranded DNA sequences
tctacccggccc

SEQ ID NO: 2 - DNA, 12 bp, Artificial Sequence
  the sequences segment associated with the vehicle surface having the sequence 5'-NH2-(CH2)6-TCTACCCGGCCC-3'.
tctacccggccc

SEQ ID NO: 3 - DNA, 28 bp, Artificial Sequence
  sequences segment of anti-VEGF aptamer
acctgggggagtattgcggaggaaggtt

SEQ ID NO: 4 - DNA, 25 bp, Artificial Sequence
  sequences segment of VEGF aptamer
tgtgggggtggacgggccgggtaga